European Patent Application EP 4 209 513 A1, published July 12, 2023. Title: Anti-VEGF-anti-PD-L1 bispecific antibody, pharmaceutical composition of same and uses thereof. Applicant: BIOTHEUS INC. The sequence listing filed with the application follows.

SEQUENCE LISTING (31 sequences)

SEQ ID NO: 1 - protein, 578 aa, Artificial Sequence
  ava-2GS-NSD HC
EVQLVESGGGLVQPGGSLRLSCAASGYTFTNYGMNWVRQAPGKGLEWVGWINTYTGEPTYAADFKRRFTFSLDTSKSTAYLQMNSLRAEDTAVYYCAKYPHYYGSSHWYFDVWGQGTLVTVSSASTKGPSVFPLAPSSKSTSGGTAALGCLVKDYFPEPVTVSWNSGALTSGVHTFPAVLQSSGLYSLSSVVTVPSSSLGTQTYICNVNHKPSNTKVDKKVEPKSCDKTHTCPPCPAPEAAGGPSVFLFPPKPKDTLMISRTPEVTCVVVDVSHEDPEVKFNWYVDGVEVHNAKTKPREEQYNSTYRVVSVLTVLHQDWLNGKEYKCKVSNKALPAPIEKTISKAKGQPREPQVYTLPPSRDELTKNQVSLTCLVKGFYPSDIAVEWESNGQPENNYKTTPPVLDSDGSFFLYSKLTVDKSRWQQGNVFSCSVMHEALHNHYTQKSLSLSPGGGGGSGGGGSGEVQLQESGGGLVQPGGSLRLSCAASGFTFSSYWMYWLRQAPGKGLEWVSSINSDSSSTYYRDSVKGRFTISRDNAKNTLYLQMNSLKSEDTAVYYCAKDPGGYAKGQGTQVTVSS

SEQ ID NO: 2 - protein, 588 aa, Artificial Sequence
  ava-4GS-NSD HC
EVQLVESGGGLVQPGGSLRLSCAASGYTFTNYGMNWVRQAPGKGLEWVGWINTYTGEPTYAADFKRRFTFSLDTSKSTAYLQMNSLRAEDTAVYYCAKYPHYYGSSHWYFDVWGQGTLVTVSSASTKGPSVFPLAPSSKSTSGGTAALGCLVKDYFPEPVTVSWNSGALTSGVHTFPAVLQSSGLYSLSSVVTVPSSSLGTQTYICNVNHKPSNTKVDKKVEPKSCDKTHTCPPCPAPEAAGGPSVFLFPPKPKDTLMISRTPEVTCVVVDVSHEDPEVKFNWYVDGVEVHNAKTKPREEQYNSTYRVVSVLTVLHQDWLNGKEYKCKVSNKALPAPIEKTISKAKGQPREPQVYTLPPSRDELTKNQVSLTCLVKGFYPSDIAVEWESNGQPENNYKTTPPVLDSDGSFFLYSKLTVDKSRWQQGNVFSCSVMHEALHNHYTQKSLSLSPGGGGGSGGGGSGGGGSGGGGSGEVQLQESGGGLVQPGGSLRLSCAASGFTFSSYWMYWLRQAPGKGLEWVSSINSDSSSTYYRDSVKGRFTISRDNAKNTLYLQMNSLKSEDTAVYYCAKDPGGYAKGQGTQVTVSS

SEQ ID NO: 3 - protein, 123 aa, Artificial Sequence [sequence omitted]

SEQ ID NO: 4 - protein, 329 aa, Artificial Sequence
  IgG1 CH(LALA)
ASTKGPSVFPLAPSSKSTSGGTAALGCLVKDYFPEPVTVSWNSGALTSGVHTFPAVLQSSGLYSLSSVVTVPSSSLGTQTYICNVNHKPSNTKVDKKVEPKSCDKTHTCPPCPAPEAAGGPSVFLFPPKPKDTLMISRTPEVTCVVVDVSHEDPEVKFNWYVDGVEVHNAKTKPREEQYNSTYRVVSVLTVLHQDWLNGKEYKCKVSNKALPAPIEKTISKAKGQPREPQVYTLPPSRDELTKNQVSLTCLVKGFYPSDIAVEWESNGQPENNYKTTPPVLDSDGSFFLYSKLTVDKSRWQQGNVFSCSVMHEALHNHYTQKSLSLSPG

SEQ ID NO: 5 - protein, 115 aa, Artificial Sequence
  VHH-C-Ye-18-5
EVQLQESGGGLVQPGGSLRLSCAASGFTFSSYWMYWLRQAPGKGLEWVSSINSDSSSTYYRDSVKGRFTISRDNAKNTLYLQMNSLKSEDTAVYYCAKDPGGYAKGQGTQVTVSS

SEQ ID NO: 6 - protein, 11 aa, Artificial Sequence
  linker G4S2
GGGGSGGGGSG

SEQ ID NO: 7 - protein, 21 aa, Artificial Sequence
  linker G4S4
GGGGSGGGGSGGGGSGGGGSG

SEQ ID NO: 8 - protein, 214 aa, Artificial Sequence
  ava-LC
DIQMTQSPSSLSASVGDRVTITCSASQDISNYLNWYQQKPGKAPKVLIYFTSSLHSGVPSRFSGSGSGTDFTLTISSLQPEDFATYYCQQYSTVPWTFGQGTKVEIKRTVAAPSVFIFPPSDEQLKSGTASVVCLLNNFYPREAKVQWKVDNALQSGNSQESVTEQDSKDSTYSLSSTLTLSKADYEKHKVYACEVTHQGLSSPVTKSFNRGEC

SEQ ID NO: 9 - protein, 107 aa, Artificial Sequence [sequence omitted]

SEQ ID NO: 10 - protein, 107 aa, Artificial Sequence [sequence omitted]

SEQ ID NO: 11 - protein, 578 aa, Artificial Sequence
  Luc-2GS-NSD HC
EVQLVESGGGLVQPGGSLRLSCAASGYDFTHYGMNWVRQAPGKGLEWVGWINTYTGEPTYAADFKRRFTFSLDTSKSTAYLQMNSLRAEDTAVYYCAKYPYYYGTSHWYFDVWGQGTLVTVSSASTKGPSVFPLAPSSKSTSGGTAALGCLVKDYFPEPVTVSWNSGALTSGVHTFPAVLQSSGLYSLSSVVTVPSSSLGTQTYICNVNHKPSNTKVDKKVEPKSCDKTHTCPPCPAPEAAGGPSVFLFPPKPKDTLMISRTPEVTCVVVDVSHEDPEVKFNWYVDGVEVHNAKTKPREEQYNSTYRVVSVLTVLHQDWLNGKEYKCKVSNKALPAPIEKTISKAKGQPREPQVYTLPPSRDELTKNQVSLTCLVKGFYPSDIAVEWESNGQPENNYKTTPPVLDSDGSFFLYSKLTVDKSRWQQGNVFSCSVMHEALHNHYTQKSLSLSPGGGGGSGGGGSGEVQLQESGGGLVQPGGSLRLSCAASGFTFSSYWMYWLRQAPGKGLEWVSSINSDSSSTYYRDSVKGRFTISRDNAKNTLYLQMNSLKSEDTAVYYCAKDPGGYAKGQGTQVTVSS

SEQ ID NO: 12 - protein, 588 aa, Artificial Sequence
  Luc-4GS-NSD HC
EVQLVESGGGLVQPGGSLRLSCAASGYDFTHYGMNWVRQAPGKGLEWVGWINTYTGEPTYAADFKRRFTFSLDTSKSTAYLQMNSLRAEDTAVYYCAKYPYYYGTSHWYFDVWGQGTLVTVSSASTKGPSVFPLAPSSKSTSGGTAALGCLVKDYFPEPVTVSWNSGALTSGVHTFPAVLQSSGLYSLSSVVTVPSSSLGTQTYICNVNHKPSNTKVDKKVEPKSCDKTHTCPPCPAPEAAGGPSVFLFPPKPKDTLMISRTPEVTCVVVDVSHEDPEVKFNWYVDGVEVHNAKTKPREEQYNSTYRVVSVLTVLHQDWLNGKEYKCKVSNKALPAPIEKTISKAKGQPREPQVYTLPPSRDELTKNQVSLTCLVKGFYPSDIAVEWESNGQPENNYKTTPPVLDSDGSFFLYSKLTVDKSRWQQGNVFSCSVMHEALHNHYTQKSLSLSPGGGGGSGGGGSGGGGSGGGGSGEVQLQESGGGLVQPGGSLRLSCAASGFTFSSYWMYWLRQAPGKGLEWVSSINSDSSSTYYRDSVKGRFTISRDNAKNTLYLQMNSLKSEDTAVYYCAKDPGGYAKGQGTQVTVSS

SEQ ID NO: 13 - protein, 123 aa, Artificial Sequence [sequence omitted]

SEQ ID NO: 14 - protein, 214 aa, Artificial Sequence
  Luc-LC
DIQLTQSPSSLSASVGDRVTITCSASQDISNYLNWYQQKPGKAPKVLIYFTSSLHSGVPSRFSGSGSGTDFTLTISSLQPEDFATYYCQQYSTVPWTFGQGTKVEIKRTVAAPSVFIFPPSDEQLKSGTASVVCLLNNFYPREAKVQWKVDNALQSGNSQESVTEQDSKDSTYSLSSTLTLSKADYEKHKVYACEVTHQGLSSPVTKSFNRGEC

SEQ ID NO: 15 - protein, 107 aa, Artificial Sequence [sequence omitted]

SEQ ID NO: 16 - protein, 567 aa, Artificial Sequence
  NSD-Elyea
EVQLQESGGGLVQPGGSLRLSCAASGFTFSSYWMYWLRQAPGKGLEWVSSINSDSSSTYYRDSVKGRFTISRDNAKNTLYLQMNSLKSEDTAVYYCAKDPGGYAKGQGTQVTVSSDKTHTCPPCPAPEAAGGPSVFLFPPKPKDTLMISRTPEVTCVVVDVSHEDPEVKFNWYVDGVEVHNAKTKPREEQYNSTYRVVSVLTVLHQDWLNGKEYKCKVSNKALPAPIEKTISKAKGQPREPQVYTLPPSRDELTKNQVSLTCLVKGFYPSDIAVEWESNGQPENNYKTTPPVLDSDGSFFLYSKLTVDKSRWQQGNVFSCSVMHEALHNHYTQKSLSLSPGGGGGSGGGGSGGGGSGGGGSGSDTGRPFVEMYSEIPEIIHMTEGRELVIPCRVTSPNITVTLKKFPLDTLIPDGKRIIWDSRKGFIISNATYKEIGLLTCEATVNGHLYKTNYLTHRQTNTIIDVVLSPSHGIELSVGEKLVLNCTARTELNVGIDFNWEYPSSKHQHKKLVNRDLKTQSGSEMKKFLSTLTIDGVTRSDQGLYTCAASSGLMTKKNSTFVRVHEK

SEQ ID NO: 17 - protein, 205 aa, Artificial Sequence
  Elyea
SDTGRPFVEMYSEIPEIIHMTEGRELVIPCRVTSPNITVTLKKFPLDTLIPDGKRIIWDSRKGFIISNATYKEIGLLTCEATVNGHLYKTNYLTHRQTNTIIDVVLSPSHGIELSVGEKLVLNCTARTELNVGIDFNWEYPSSKHQHKKLVNRDLKTQSGSEMKKFLSTLTIDGVTRSDQGLYTCAASSGLMTKKNSTFVRVHEK

SEQ ID NO: 18 - protein, 226 aa, Artificial Sequence
  Fc(LALA)
DKTHTCPPCPAPEAAGGPSVFLFPPKPKDTLMISRTPEVTCVVVDVSHEDPEVKFNWYVDGVEVHNAKTKPREEQYNSTYRVVSVLTVLHQDWLNGKEYKCKVSNKALPAPIEKTISKAKGQPREPQVYTLPPSRDELTKNQVSLTCLVKGFYPSDIAVEWESNGQPENNYKTTPPVLDSDGSFFLYSKLTVDKSRWQQGNVFSCSVMHEALHNHYTQKSLSLSPG

SEQ ID NO: 19 - protein, 567 aa, Artificial Sequence
  Elyea-NSD
SDTGRPFVEMYSEIPEIIHMTEGRELVIPCRVTSPNITVTLKKFPLDTLIPDGKRIIWDSRKGFIISNATYKEIGLLTCEATVNGHLYKTNYLTHRQTNTIIDVVLSPSHGIELSVGEKLVLNCTARTELNVGIDFNWEYPSSKHQHKKLVNRDLKTQSGSEMKKFLSTLTIDGVTRSDQGLYTCAASSGLMTKKNSTFVRVHEKDKTHTCPPCPAPEAAGGPSVFLFPPKPKDTLMISRTPEVTCVVVDVSHEDPEVKFNWYVDGVEVHNAKTKPREEQYNSTYRVVSVLTVLHQDWLNGKEYKCKVSNKALPAPIEKTISKAKGQPREPQVYTLPPSRDELTKNQVSLTCLVKGFYPSDIAVEWESNGQPENNYKTTPPVLDSDGSFFLYSKLTVDKSRWQQGNVFSCSVMHEALHNHYTQKSLSLSPGGGGGSGGGGSGGGGSGGGGSGEVQLQESGGGLVQPGGSLRLSCAASGFTFSSYWMYWLRQAPGKGLEWVSSINSDSSSTYYRDSVKGRFTISRDNAKNTLYLQMNSLKSEDTAVYYCAKDPGGYAKGQGTQVTVSS

SEQ ID NO: 20 - protein, 108 aa, Artificial Sequence
  CH1
ASTKGPSVFPLAPSSKSTSGGTAALGCLVKDYFPEPVTVSWNSGALTSGVHTFPAVLQSSGLYSLSSVVTVPSSSLGTQTYICNVNHKPSNTKVDKKVEPKSCDKTHT

SEQ ID NO: 21 - protein, 8 aa, Artificial Sequence
  Bevacizumab-HCDR1
GYTFTNYG

SEQ ID NO: 22 - protein, 9 aa, Artificial Sequence
  Bevacizumab-HCDR2
INTYTGEPT

SEQ ID NO: 23 - protein, 16 aa, Artificial Sequence
  Bevacizumab-HCDR3
AKYPHYYGSSHWYFDV

SEQ ID NO: 24 - protein, 6 aa, Artificial Sequence
  Bevacizumab-LCDR1
QDISNY

SEQ ID NO: 25 - protein, 3 aa, Artificial Sequence
  Bevacizumab-LCDR2
FTS

SEQ ID NO: 26 - protein, 9 aa, Artificial Sequence
  Bevacizumab-LCDR3
QQYSTVPWT

SEQ ID NO: 27 - protein, 8 aa, Artificial Sequence
  Ranibizumab-HCDR1
GYDFTHYG

SEQ ID NO: 28 - protein, 16 aa, Artificial Sequence
  Ranibizumab-HCDR3
AKYPYYYGTSHWYFDV

SEQ ID NO: 29 - protein, 8 aa, Artificial Sequence
  HCDR1 of C-Ye-18-5 VH
GFTFSSYW

SEQ ID NO: 30 - protein, 8 aa, Artificial Sequence
  HCDR2 of C-Ye-18-5 VH
INSDSSST

SEQ ID NO: 31 - protein, 8 aa, Artificial Sequence
  HCDR3 of C-Ye-18-5 VH
AKDPGGYA